European Patent Application EP 4 442 824 A1, published October 9, 2024. Title: 結合物質及び分析方法. Applicant: DENSO CORPORATION. The sequence listing filed with the application follows.

SEQUENCE LISTING (6 sequences)

SEQ ID NO: 1 - DNA, 78 bp, synthetic construct
  source 1..78: mol_type = other DNA
ttttttcagcaccgaccttgtgctttgggagtgctggtccaagggcgttaatggacattttctacatctcagcattct

SEQ ID NO: 2 - DNA, 51 bp, synthetic construct
  source 1..51: mol_type = other DNA
cagcaccgaccttgtgctttgggagtgctggtccaagggcgttaatggaca

SEQ ID NO: 3 - DNA, 15 bp, synthetic construct
  source 1..15: mol_type = other DNA
acatctcagcattct

SEQ ID NO: 4 - DNA, 29 bp, synthetic construct
  source 1..29: mol_type = other DNA
aatggacattttctacatctcagcattct

SEQ ID NO: 5 - DNA, 29 bp, synthetic construct
  source 1..29: mol_type = other DNA
agaatgctgagatgtagaaaatgtccatt

SEQ ID NO: 6 - DNA, 75 bp, synthetic construct
  source 1..75: mol_type = other DNA
gagatgtaccacgaggaaactgtgaagatcgcttcacgagcaacatgaagattgtaggtcacgagtcagaatgct